European Patent Specification EP 3 999 095 B1, published September 13, 2023. Title: METHOD FOR TREATING SARCOIDOSIS. Applicant: University of Miami. The sequence listing filed with the application follows.

SEQUENCE LISTING (8 sequences)

SEQ ID NO: 1 - protein, 29 aa, Homo sapiens
  MISC_FEATURE: hGHRH (1-29)HN2
YADAIFTNSYRKVLGQLSARKLLQDIMSR

SEQ ID NO: 2 - protein, 32 aa, Artificial Sequence
  Synthetic Polypeptide
  MISC_FEATURE (1)..(1): Xaa is PhAc (phenylacetyl), Nac (naphthylacetyl), Oct (octanoyl), N-Me-Aib (N-methyl-alpha-aminoisobutyroyl), Dca (dichloroacetyl), Ac-Ada (acetyl-12-aminododecanoyl), Fer (ferulyl), Ac-Amc (acetyl-8-aminocaprylyl), Me-NH-Sub (methyl-NH-suberyl),
  MISC_FEATURE (3)..(3): Xaa is D-Arg
  MISC_FEATURE (5)..(5): Xaa is Ala or Me-Ala
  MISC_FEATURE (7)..(7): Xaa is Cpa (para-chlorophenylalanine) or Phe(F)
  MISC_FEATURE (9)..(9): Xaa is Ala, Pal (pyridylalanine), Dip ((3,3-diphenyl)alanine), or Me-Ala
  MISC_FEATURE (10)..(10): Xaa is Har
  MISC_FEATURE (11)..(11): Xaa is FPa5, Tyr(Alk) where Alk is Me or Et
  MISC_FEATURE (12)..(12): Xaa is His or Arg
  MISC_FEATURE (13)..(13): Xaa is Lys, Lys(0-11) (Lys(A0-A1-A2-A3-A4-A5-A6-A7-A8-A9 A10-A11-), Lys(Me)2, or Orn (ornithine)
  MISC_FEATURE (16)..(16): Xaa is Abu (alpha-aminobutyric acid) or Orn
  MISC_FEATURE (18)..(18): Xaa is Leu or Glu
  MISC_FEATURE (21)..(21): Xaa is Har (homoarginine) or His
  MISC_FEATURE (22)..(22): Xaa is Lys, Lys(Me)2 or Orn
  MISC_FEATURE (28)..(28): Xaa is Nle
  MISC_FEATURE (29)..(29): Xaa is D-Arg
  MISC_FEATURE (30)..(30): Xaa is Har, Arg or Agm (agmatine)
  MISC_FEATURE (31)..(31): Xaa is  Ala, Amc, Apa, Ada, AE2A , AE4P,E -Lys( alpha-NH2), Agm, or absent
  MISC_FEATURE (32)..(32): Xaa is  Lys(Oct), Ahx (6-aminohexanoyl), or absent
  MOD_RES (32)..(32): AMIDATION
XYXDXIXTXXXXXVLXQXSAXXLLQDIXXXXX

SEQ ID NO: 3 - protein, 32 aa, Artificial Sequence
  Synthetic Polypeptide
  MISC_FEATURE (1)..(1): Xaa is Phac
  MISC_FEATURE (2)..(2): Xaa is Ada
  MISC_FEATURE (4)..(4): Xaa is D-Arg
  MISC_FEATURE (8)..(8): Xaa is Phe(F)5
  MISC_FEATURE (11)..(11): Xaa is Har
  MISC_FEATURE (12)..(12): Xaa is Tyr(Me)
  MISC_FEATURE (14)..(14): Xaa is Orn
  MISC_FEATURE (17)..(17): Xaa is Abu
  MISC_FEATURE (23)..(23): Xaa is Orn
  MISC_FEATURE (29)..(29): Xaa is Nle
  MISC_FEATURE (30)..(30): Xaa is D-Arg
  MISC_FEATURE (31)..(31): Xaa is Har
  MISC_FEATURE (32)..(32): Xaa is Agm
  MOD_RES (32)..(32): AMIDATION
XXYXDAIXTAXXHXVLXQLSAHXLLQDIXXXX

SEQ ID NO: 4 - protein, 32 aa, Artificial Sequence
  Synthetic Polypeptide
  MISC_FEATURE (1)..(1): Xaa is Phac
  MISC_FEATURE (2)..(2): Xaa is Ada
  MISC_FEATURE (4)..(4): Xaa is D-Arg
  MISC_FEATURE (8)..(8): Xaa is Phe(F)5
  MISC_FEATURE (9)..(9): Xaa is Thr(Me)
  MISC_FEATURE (11)..(11): Xaa is Har
  MISC_FEATURE (12)..(12): Xaa is Tyr(Me)
  MISC_FEATURE (14)..(14): Xaa is Orn
  MISC_FEATURE (17)..(17): Xaa is Abu
  MISC_FEATURE (23)..(23): Xaa is Orn
  MISC_FEATURE (29)..(29): Xaa is Nle
  MISC_FEATURE (30)..(30): Xaa is D-Arg
  MISC_FEATURE (31)..(31): Xaa is Har
  MISC_FEATURE (32)..(32): Xaa is Agm
  MOD_RES (32)..(32): AMIDATION
XXYXDAIXXAXXHXVLXQLSAHXLLQDIXXXX

SEQ ID NO: 5 - protein, 31 aa, Artificial Sequence
  Synthetic Polypeptide
  MISC_FEATURE (1)..(1): Xaa is Phac
  MISC_FEATURE (3)..(3): Xaa is D-Ala
  MISC_FEATURE (7)..(7): Xaa is Cpa
  MISC_FEATURE (10)..(10): Xaa is Har
  MISC_FEATURE (11)..(11): Xaa is Fpa
  MISC_FEATURE (13)..(13): Xaa is Orn
  MISC_FEATURE (16)..(16): Xaa is Abu
  MISC_FEATURE (22)..(22): Xaa is Orn
  MISC_FEATURE (28)..(28): Xaa is Nle
  MISC_FEATURE (29)..(29): Xaa is D-Arg
  MISC_FEATURE (30)..(30): Xaa is Har
  MISC_FEATURE (31)..(31): Xaa is Ada
  MOD_RES (31)..(31): AMIDATION
XYXDAIXTAXXHXVLXQLSAHXLLGAIXXXX

SEQ ID NO: 6 - protein, 32 aa, Artificial Sequence
  Synthetic Polypeptide
  MISC_FEATURE (1)..(1): Xaa is Phac
  MISC_FEATURE (2)..(2): Xaa is Ada
  MISC_FEATURE (4)..(4): Xaa is D-Arg
  MISC_FEATURE (8)..(8): Xaa is Cpa
  MISC_FEATURE (11)..(11): Xaa is Har
  MISC_FEATURE (12)..(12): Xaa is Fpa
  MISC_FEATURE (14)..(14): Xaa is Orn
  MISC_FEATURE (17)..(17): Xaa is Abu
  MISC_FEATURE (23)..(23): Xaa is Orn
  MISC_FEATURE (29)..(29): Xaa is Nle
  MISC_FEATURE (30)..(30): Xaa is D-Arg
  MISC_FEATURE (31)..(31): Xaa is Har
  MISC_FEATURE (32)..(32): Xaa is Ada
  MISC_FEATURE (32)..(32): C-Term NH2
  MOD_RES (32)..(32): AMIDATION
XXYXDAIXTAXXHXVLXQQSAHXLLQDIXXXX

SEQ ID NO: 7 - protein, 31 aa, Artificial Sequence
  Synthetic Polypeptide
  MISC_FEATURE (1)..(1): Xaa is Phac
  MISC_FEATURE (2)..(2): Xaa is Ada
  MISC_FEATURE (4)..(4): Xaa is D-Arg
  MISC_FEATURE (8)..(8): Xaa is Cpa
  MISC_FEATURE (11)..(11): Xaa is Har
  MISC_FEATURE (12)..(12): Xaa is Fpa
  MISC_FEATURE (14)..(14): Xaa is Orn
  MISC_FEATURE (17)..(17): Xaa is Abu
  MISC_FEATURE (23)..(23): Xaa is Orn
  MISC_FEATURE (29)..(29): Xaa is Nle
  MISC_FEATURE (30)..(30): Xaa is D-Arg
  MISC_FEATURE (31)..(31): Xaa is Har
  MOD_RES (31)..(31): AMIDATION
XXYXDAIXTAXXHXVLXQLSAHXLLQDIXXX

SEQ ID NO: 8 - protein, 31 aa, Artificial Sequence
  Synthetic Polypeptide
  MISC_FEATURE (1)..(1): Xaa is PhAc
  MISC_FEATURE (2)..(2): Xaa is Ada
  MISC_FEATURE (4)..(4): Xaa is D-ARg
  MISC_FEATURE (8)..(8): Xaa is Fpa
  MISC_FEATURE (11)..(11): Xaa is Har
  MISC_FEATURE (12)..(12): Xaa is Tyr(Me)
  MISC_FEATURE (14)..(14): Xaa is Orn
  MISC_FEATURE (17)..(17): Xaa is Abu
  MISC_FEATURE (22)..(22): Xaa is Orn
  MISC_FEATURE (29)..(29): Xaa is Nle
  MISC_FEATURE (30)..(30): Xaa is D-Arg
  MISC_FEATURE (31)..(31): Xaa is Har
XXYXDAIXTAXXHXVLXQLSAXKLLQDIXXX